European Patent Specification EP 3 922 259 B1, published April 1, 2026. Title: METHODS AND COMPOSITIONS USING GDF15 POLYPEPTIDES FOR INCREASING RED BLOOD CELLS. Applicant: ACCELERON PHARMA INC. The sequence listing filed with the application follows.

SEQUENCE LISTING (15 sequences)

SEQ ID NO: 1 - protein, 308 aa, Homo sapiens
MPGQELRTVNGSQMLLVLLVLSWLPHGGALSLAEASRASFPGPSELHSEDSRFRELRKRYEDLLTRLRANQSWEDSNTDLVPAPAVRILTPEVRLGSGGHLHLRISRAALPEGLPEASRLHRALFRLSPTASRSWDVTRPLRRQLSLARPQAPALHLRLSPPPSQSDQLLAESSSARPQLELHLRPQAARGRRRARARNGDHCPLGPGRCCRLHTVRASLEDLGWADWVLSPREVQVTMCIGACPSQFRAANMHAQIKTSLHRLKPDTVPAPCCVPASYNPMVLIQKTDTGVSLQTYDDLLAKDCHCI

SEQ ID NO: 2 - protein, 279 aa, Homo sapiens
LSLAEASRASFPGPSELHSEDSRFRELRKRYEDLLTRLRANQSWEDSNTDLVPAPAVRILTPEVRLGSGGHLHLRISRAALPEGLPEASRLHRALFRLSPTASRSWDVTRPLRRQLSLARPQAPALHLRLSPPPSQSDQLLAESSSARPQLELHLRPQAARGRRRARARNGDHCPLGPGRCCRLHTVRASLEDLGWADWVLSPREVQVTMCIGACPSQFRAANMHAQIKTSLHRLKPDTVPAPCCVPASYNPMVLIQKTDTGVSLQTYDDLLAKDCHCI

SEQ ID NO: 3 - protein, 112 aa, Homo sapiens
ARNGDHCPLGPGRCCRLHTVRASLEDLGWADWVLSPREVQVTMCIGACPSQFRAANMHAQIKTSLHRLKPDTVPAPCCVPASYNPMVLIQKTDTGVSLQTYDDLLAKDCHCI

SEQ ID NO: 4 - protein, 110 aa, Homo sapiens
NGDHCPLGPGRCCRLHTVRASLEDLGWADWVLSPREVQVTMCIGACPSQFRAANMHAQIKTSLHRLKPDTVPAPCCVPASYNPMVLIQKTDTGVSLQTYDDLLAKDCHCI

SEQ ID NO: 5 - protein, 110 aa, Artificial Sequence
  source: /note="Description of Artificial Sequence: Synthetic polypeptide"
QGDHCPLGPGRCCRLHTVRASLEDLGWADWVLSPREVQVTMCIGACPSQFRAANMHAQIKTSLHRLKPDTVPAPCCVPASYNPMVLIQKTDTGVSLQTYDDLLAKDCHCI

SEQ ID NO: 6 - protein, 110 aa, Artificial Sequence
  source: /note="Description of Artificial Sequence: Synthetic polypeptide"
NGDDCPLGPGRCCRLHTVRASLEDLGWADWVLSPREVQVTMCIGACPSQFRAANMHAQIKTSLHRLKPDTVPAPCCVPASYNPMVLIQKTDTGVSLQTYDDLLAKDCHCI

SEQ ID NO: 7 - protein, 110 aa, Artificial Sequence
  source: /note="Description of Artificial Sequence: Synthetic polypeptide"
QGDDCPLGPGRCCRLHTVRASLEDLGWADWVLSPREVQVTMCIGACPSQFRAANMHAQIKTSLHRLKPDTVPAPCCVPASYNPMVLIQKTDTGVSLQTYDDLLAKDCHCI

SEQ ID NO: 8 - protein, 108 aa, Artificial Sequence
  source: /note="Description of Artificial Sequence: Synthetic polypeptide"
DHCPLGPGRCCRLHTVRASLEDLGWADWVLSPREVQVTMCIGACPSQFRAANMHAQIKTSLHRLKPDTVPAPCCVPASYNPMVLIQKTDTGVSLQTYDDLLAKDCHCI

SEQ ID NO: 9 - protein, 108 aa, Artificial Sequence
  source: /note="Description of Artificial Sequence: Synthetic polypeptide"
DDCPLGPGRCCRLHTVRASLEDLGWADWVLSPREVQVTMCIGACPSQFRAANMHAQIKTSLHRLKPDTVPAPCCVPASYNPMVLIQKTDTGVSLQTYDDLLAKDCHCI

SEQ ID NO: 10 - protein, 303 aa, Mus musculus
MAPPALQAQPPGGSQLRFLLFLLLLLLLLSWPSQGDALAMPEQRPSGPESQLNADELRGRFQDLLSRLHANQSREDSNSEPSPDPAVRILSPEVRLGSHGQLLLRVNRASLSQGLPEAYRVHRALLLLTPTARPWDITRPLKRALSLRGPRAPALRLRLTPPPDLAMLPSGGTQLELRLRVAAGRGRRSAHAHPRDSCPLGPGRCCHLETVQATLEDLGWSDWVLSPRQLQLSMCVGECPHLYRSANTHAQIKARLHGLQPDKVPAPCCVPSSYTPVVLMHRTDSGVSLQTYDDLVARGCHCA

SEQ ID NO: 11 - protein, 112 aa, Mus musculus
AHPRDSCPLGPGRCCHLETVQATLEDLGWSDWVLSPRQLQLSMCVGECPHLYRSANTHAQIKARLHGLQPDKVPAPCCVPSSYTPVVLMHRTDSGVSLQTYDDLVARGCHCA

SEQ ID NO: 12 - protein, 108 aa, Artificial Sequence
  source: /note="Description of Artificial Sequence: Synthetic polypeptide"
DSCPLGPGRCCHLETVQATLEDLGWSDWVLSPRQLQLSMCVGECPHLYRSANTHAQIKARLHGLQPDKVPAPCCVPSSYTPVVLMHRTDSGVSLQTYDDLVARGCHCA

SEQ ID NO: 13 - DNA, 924 bp, Homo sapiens
atgcccgggcaagaactcaggacggtgaatggctctcagatgctcctggtgttgctggtgctctcgtggctgccgcatgggggcgccctgtctctggccgaggcgagccgcgcaagtttcccgggaccctcagagttgcactccgaagactccagattccgagagttgcggaaacgctacgaggacctgctaaccaggctgcgggccaaccagagctgggaagattcgaacaccgacctcgtcccggcccctgcagtccggatactcacgccagaagtgcggctgggatccggcggccacctgcacctgcgtatctctcgggccgcccttcccgaggggctccccgaggcctcccgccttcaccgggctctgttccggctgtccccgacggcgtcaaggtcgtgggacgtgacacgaccgctgcggcgtcagctcagccttgcaagaccccaggcacccgcgctgcacctgcgactgtcgccgccgccgtcgcagtcggaccaactgctggcagaatcttcgtccgcacggccccagctggagttgcacttgcggccgcaagccgccagggggcgccgcagagcgcgtgcgcgcaacggggaccactgtccgctcgggcccgggcgttgctgccgtctgcacacggtccgcgcgtcgctggaagacctgggctgggccgattgggtgctgtcgccacgggaggtgcaagtgaccatgtgcatcggcgcgtgcccgagccagttccgggcggcaaacatgcacgcgcagatcaagacgagcctgcaccgcctgaagcccgacacggtgccagcgccctgctgcgtgcccgccagctacaatcccatggtgctcattcaaaagaccgacaccggggtgtcactccagacctatgatgacttgttagccaaagactgccactgcata

SEQ ID NO: 14 - DNA, 909 bp, Mus musculus
atggccccgcccgcgctccaggcccagcctccaggcggctctcaactgaggttcctgctgttcctgctgctgttgctgctgctgctgtcatggccatcgcagggggacgccctggcaatgcctgaacagcgaccctccggccctgagtcccaactcaacgccgacgagctacggggtcgcttccaggacctgctgagccggctgcatgccaaccagagccgagaggactcgaactcagaaccaagtcctgacccagctgtccggatactcagtccagaggtgagattggggtcccacggccagctgctactccgcgtcaaccgggcgtcgctgagtcagggtctccccgaagcctaccgcgtgcaccgagcgctgctcctgctgacgccgacggcccgcccctgggacatcactaggcccctgaagcgtgcgctcagcctccggggaccccgtgctcccgcattacgcctgcgcctgacgccgcctccggacctggctatgctgccctctggcggcacgcagctggaactgcgcttacgggtagccgccggcagggggcgccgaagcgcgcatgcgcacccaagagactcgtgcccactgggtccagggcgctgctgtcacttggagactgtgcaggcaactcttgaagacttgggctggagcgactgggtgctgtccccgcgccagctgcagctgagcatgtgcgtgggcgagtgtccccacctgtatcgctccgcgaacacgcatgcgcagatcaaagcacgcctgcatggcctgcagcctgacaaggtgcctgccccgtgctgtgtcccctccagctacaccccggtggttcttatgcacaggacagacagtggtgtgtcactgcagacttatgatgacctggtggcccggggctgccactgcgct

SEQ ID NO: 15 - protein, 6 aa, Artificial Sequence
  source: /note="Description of Artificial Sequence: Synthetic 6xHis tag"
HHHHHH